European Patent Specification EP 3 382 020 B1, published January 24, 2024. Title: Expression vector and lipid membrane structure encapsulating the vector. Applicant: National University Corporation Hokkaido University. The sequence listing filed with the application follows.

SEQUENCE LISTING (13 sequences)

SEQ ID NO: 1 - DNA, 2645 bp, Artificial Sequence
  CDS (583)..(2499): Recombinant DNA comprising CMV promoter sequence,ND4 coding sequence, FLAG Tag sequence, Luciferase coding sequence and mitochondrial tRNA-Asp sequence
ctgcagattaatagtaatcaattacggggtcattagttcatagcccatatatggagttccgcgttacataacttacggtaaatggcccgcctggctgaccgcccaacgacccccgcccattgacgtcaataatgacgtatgttcccatagtaacgccaatagggactttccattgacgtcaatgggtggagtatttacggtaaactgcccacttggcagtacatcaagtgtatcatatgccaagtccgccccctattgacgtcaatgacggtaaatggcccgcctggcattatgcccagtacatgaccttacgggactttcctacttggcagtacatctacgtattagtcatcgctattaccatgctgatgcggttttggcagtacaccaatgggcgtggatagcggtttgactcacggggatttccaagtctccaccccattgacgtcaatgggagtttgttttggcaccaaaatcaacgggactttccaaaatgtcgtaataaccccgccccgttgacgcaaatgggcggtaggcgtgtacggtgggaggtctatataagcagacgtcgtttagtgaaccatgctaaaaattattcttccctcactaatgctactaccactaacctgactatcaagccctaaaaaaacctgaacaaacgtaacctcatatagttttctaattagtttaaccagcctaacacttctatgacaaaccgacgaaaattataaaaacttttcaaatatattctcctcagaccccctatccacaccattaattattttaacagcctgattactgccactaatattaatagctagccaaaaccacctaaaaaaagataataacgtactacaaaaactctacatctcaatactaatcagcttacaaattctcctaatcataaccttttcagcaactgaactaattatattttatattttatttgaagcaaccttaatcccaacacttattattattacccgatgagggaaccaaactgaacgcctaaacgcagggatttatttcctattttataccctaatcggttctattccactgctaattgccctcatcttaatccaaaaccatgtaggaaccctaaacctcataattttatcattcacaacacacaccttagacgcttcatgatctaacaacttactatggttggcatgcataatagcatttcttattaaaataccattatatggagttcacctatgactaccaaaagcccatgttgaagctccaattgctgggtcaataattctagcagctattcttctaaaattaggtagttacggaataattcgcatctccattattctagacccactaacaaaatatatagcataccccttcatccttctctccctatgaggaataattataactagctcaatctgcttacgccaaacagatttaaaatcactaatcgcctactcctcagttagccacatagcacttgttattgcatcaatcataatccaaactccatgaagcttcataggagcaacaatactaataatcgcacatggcctcacatcatcactcctattctgcctagcaaactccaactacgaacggatccacagccgtactataatcatggcccgaggacttcaaatggtcttcccacttatagccacatgatgactgatagcaagtctagctaatctagctctacccccttcaatcaatctaataggagaattattcattaccatatcattattttcttgatcaaactttaccattattcttataggaattaacattattattacaggtatatactcaatatacataattattaccacccaacgcggcaaactaaccaaccatataattaacctccaaccctcacacacacgagaactaacactaatagcccttcacataattccacttattcttctaactaccaatccaaaactaattacaggcctgacaatagattacaaggatgacgacgataagatggtcttcacactcgaagatttcgttggggactgacgacagacagccggctacaacctggaccaagtccttgaacagggaggtgtgtccagtttgtttcagaatctcggggtgtccgtaactccgatccaacggattgtcctgagcggtgaaaatgggctgaagatcgacatccatgtcatcatcccgtatgaaggtctgagcggcgaccaaatgggccagatcgaaaaaatttttaaggtggtgtaccctgtggatgatcatcactttaaggtgatcctgcactatggcacactggtaatcgacggggttacgccgaacatgatcgactatttcggacggccgtatgaaggcatcgccgtgttcgacggcaaaaagatcactgtaacagggaccctgtggaacggcaacaaaattatcgacgagcgcctgatcaaccccgacggctccctgctgttccgagtaaccatcaacggagtgaccggctggcggctgtgcgaacgcattctggcgtaagaaaggaaggaatcgaaccccctaaaattggtttcaagccaatctcatatcctatatgtctttctcaataagatattagtaaaatcaattacataactttgtcaaagttaaattatagatcaataatctatatatcttatctgcag

SEQ ID NO: 2 - protein, 638 aa, Artificial sequence
  Fusion protein consisting of ND4, FLAG tag and Luciferase
MLKIILPSLMLLPLTWLSSPKKTWTNVTSYSFLISLTSLTLLWQTDENYKNFSNIFSSDPLSTPLIILTAWLLPLILIASQNHLKKDNNVLQKLYISILISLQILLIITFSATELIIFYILFEATLIPTLIIITRWGNQTERLNAGIYFLFYTLIGSIPLLIALILIQNHVGTLNLIILSFTTHTLDASWSNNLLWLACIIAFLIKIPLYGVHLWLPKAHVEAPIAGSIILAAILLKLGSYGIIRISIILDPLTKYIAYPFILLSLWGIIITSSICLRQTDLKSLIAYSSVSHIALVIASIIIQTPWSFIGATILIIAHGLTSSLLFCLANSNYERIHSRTIIMARGLQMVFPLIATWWLIASLANLALPPSINLIGELFITISLFSWSNFTIILIGINIIITGIYSIYIIITTQRGKLTNHIINLQPSHTRELTLIALHIIPLILLTTNPKLITGLTIDYKDDDDKMVFTLEDFVGDWRQTAGYNLDQVLEQGGVSSLFQNLGVSVTPIQRIVLSGENGLKIDIHVIIPYEGLSGDQMGQIEKIFKVVYPVDDHHFKVILHYGTLVIDGVTPNMIDYFGRPYEGIAVFDGKKITVTGTLWNGNKIIDERLINPDGSLLFRVTINGVTGWRLCERILA

SEQ ID NO: 3 - DNA, 2645 bp, Artificial sequence
  CDS (583)..(2499): Recombinant DNA comprising CMV promoter sequence,ND4 coding sequence, FLAG Tag sequence, Luciferase coding sequence and mitochondrial tRNA-Asp sequence
ctgcagattaatagtaatcaattacggggtcattagttcatagcccatatatggagttccgcgttacataacttacggtaaatggcccgcctggctgaccgcccaacgacccccgcccattgacgtcaataatgacgtatgttcccatagtaacgccaatagggactttccattgacgtcaatgggtggagtatttacggtaaactgcccacttggcagtacatcaagtgtatcatatgccaagtccgccccctattgacgtcaatgacggtaaatggcccgcctggcattatgcccagtacatgaccttacgggactttcctacttggcagtacatctacgtattagtcatcgctattaccatgctgatgcggttttggcagtacaccaatgggcgtggatagcggtttgactcacggggatttccaagtctccaccccattgacgtcaatgggagtttgttttggcaccaaaatcaacgggactttccaaaatgtcgtaataaccccgccccgttgacgcaaatgggcggtaggcgtgtacggtgggaggtctatataagcagacgtcgtttagtgaaccatgctaaaaattattcttccctcactaatgctactaccactaacctgactatcaagccctaaaaaaacctgaacaaacgtaacctcatatagttttctaattagtttaaccagcctaacacttctatgacaaaccgacgaaaattataaaaacttttcaaatatattctcctcagaccccctatccacaccattaattattttaacagcctgattactgccactaatattaatagctagccaaaaccacctaaaaaaagataataacgtactacaaaaactctacatctcaatactaatcagcttacaaattctcctaatcataaccttttcagcaactgaactaattatattttatattttatttgaagcaaccttaatcccaacacttattattattacccgatgagggaaccaaactgaacgcctaaacgcagggatttatttcctattttataccctaatcggttctattccactgctaattgccctcatcttaatccaaaaccatgtaggaaccctaaacctcataattttatcattcacaacacacaccttagacgcttcatgatctaacaacttactatggttggcatgcataatagcatttcttattaaaataccattatatggagttcacctatgactaccaaaagcccatgttgaagctccaattgctgggtcaataattctagcagctattcttctaaaattaggtagttacggaataattcgcatctccattattctagacccactaacaaaatatatagcataccccttcatccttctctccctatgaggaataattataactagctcaatctgcttacgccaaacagatttaaaatcactaatcgcctactcctcagttagccacatagcacttgttattgcatcaatcataatccaaactccatgaagcttcataggagcaacaatactaataatcgcacatggcctcacatcatcactcctattctgcctagcaaactccaactacgaacggatccacagccgtactataatcatggcccgaggacttcaaatggtcttcccacttatagccacatgatgactgatagcaagtctagctaatctagctctacccccttcaatcaatctaataggagaattattcattaccatatcattattttcttgatcaaactttaccattattcttataggaattaacattattattacaggtatatactcaatatacataattattaccacccaacgcggcaaactaaccaaccatataattaacctccaaccctcacacacacgagaactaacactaatagcccttcacataattccacttattcttctaactaccaatccaaaactaattacaggcctgacaatagattacaaggatgacgacgataagatggtcttcacactcgaagatttcgttggggactgacgacagacagccggctacaacctggaccaagtccttgaacagggaggtgtgtccagtttgtttcagaatctcggggtgtccgtaactccgatccaacggattgtcctgagcggtgaaaatgggctgaagatcgacatccatgtcatcatcccgtatgaaggtctgagcggcgaccaaatgggccagatcgaaaaaatttttaaggtggtgtaccctgtggatgatcatcactttaaggtgatcctgcactatggcacactggtaatcgacggggttacgccgaacatgatcgactatttcggacggccgtatgaaggcatcgccgtgttcgacggcaaaaagatcactgtaacagggaccctgtgaaacggcaacaaaattatcgacgagcgcctgatcaaccccgacggctccctgctgttccgagtaaccatcaacggagtgaccggctgacggctgtgcgaacgcattctggcgtaagaaaggaaggaatcgaaccccctaaaattggtttcaagccaatctcatatcctatatgtctttctcaataagatattagtaaaatcaattacataactttgtcaaagttaaattatagatcaataatctatatatcttatctgcag

SEQ ID NO: 4 - protein, 638 aa, Artificial sequence; identical to SEQ ID NO: 2
  Fusion protein consisting of ND4, FLAG tag and Luciferase

SEQ ID NO: 5 - DNA, 2645 bp, artificial sequence
  CDS (583)..(2118): Recombinant DNA comprising CMV promoter sequence, ND4 coding sequence, FLAG Tag sequence, Luciferase coding sequence and mitochondrial tRNA-Asp sequence
ctgcagattaatagtaatcaattacggggtcattagttcatagcccatatatggagttccgcgttacataacttacggtaaatggcccgcctggctgaccgcccaacgacccccgcccattgacgtcaataatgacgtatgttcccatagtaacgccaatagggactttccattgacgtcaatgggtggagtatttacggtaaactgcccacttggcagtacatcaagtgtatcatatgccaagtccgccccctattgacgtcaatgacggtaaatggcccgcctggcattatgcccagtacatgaccttacgggactttcctacttggcagtacatctacgtattagtcatcgctattaccatgctgatgcggttttggcagtacaccaatgggcgtggatagcggtttgactcacggggatttccaagtctccaccccattgacgtcaatgggagtttgttttggcaccaaaatcaacgggactttccaaaatgtcgtaataaccccgccccgttgacgcaaatgggcggtaggcgtgtacggtgggaggtctatataagcagacgtcgtttagtgaaccatgctaaaaattattcttccctcactaatgctactaccactaacctgactatcaagccctaaaaaaacctgaacaaacgtaacctcatatagttttctaattagtttaaccagcctaacacttctatgacaaaccgacgaaaattataaaaacttttcaaatatattctcctcagaccccctatccacaccattaattattttaacagcctgattactgccactaatattaatagctagccaaaaccacctaaaaaaagataataacgtactacaaaaactctacatctcaatactaatcagcttacaaattctcctaatcataaccttttcagcaactgaactaattatattttatattttatttgaagcaaccttaatcccaacacttattattattacccgatgagggaaccaaactgaacgcctaaacgcagggatttatttcctattttataccctaatcggttctattccactgctaattgccctcatcttaatccaaaaccatgtaggaaccctaaacctcataattttatcattcacaacacacaccttagacgcttcatgatctaacaacttactatggttggcatgcataatagcatttcttattaaaataccattatatggagttcacctatgactaccaaaagcccatgttgaagctccaattgctgggtcaataattctagcagctattcttctaaaattaggtagttacggaataattcgcatctccattattctagacccactaacaaaatatatagcataccccttcatccttctctccctatgaggaataattataactagctcaatctgcttacgccaaacagatttaaaatcactaatcgcctactcctcagttagccacatagcacttgttattgcatcaatcataatccaaactccatgaagcttcataggagcaacaatactaataatcgcacatggcctcacatcatcactcctattctgcctagcaaactccaactacgaacggatccacagccgtactataatcatggcccgaggacttcaaatggtcttcccacttatagccacatgatgactgatagcaagtctagctaatctagctctacccccttcaatcaatctaataggagaattattcattaccatatcattattttcttgatcaaactttaccattattcttataggaattaacattattattacaggtatatactcaatatacataattattaccacccaacgcggcaaactaaccaaccatataattaacctccaaccctcacacacacgagaactaacactaatagcccttcacataattccacttattcttctaactaccaatccaaaactaattacaggcctgacaatagattacaaggatgacgacgataagatggtcttcacactcgaagatttcgttggggactgacgacagacagccggctacaacctggaccaagtccttgaacagggaggtgtgtccagtttgtttcagaatctcggggtgtccgtaactccgatccaatagattgtcctgagcggtgaaaatgggctgaagatcgacatccatgtcatcatcccgtatgaaggtctgagcggcgaccaaatgggccagatcgaaaaaatttttaaggtggtgtaccctgtggatgatcatcactttaaggtgatcctgcactatggcacactggtaatcgacggggttacgccgaacatgatcgactatttcggacggccgtatgaaggcatcgccgtgttcgacggcaaaaagatcactgtaacagggaccctgtggaacggcaacaaaattatcgacgagcgcctgatcaaccccgacggctccctgctgttccgagtaaccatcaacggagtgaccggctggcggctgtgcgaacgcattctggcgtaagaaaggaaggaatcgaaccccctaaaattggtttcaagccaatctcatatcctatatgtctttctcaataagatattagtaaaatcaattacataactttgtcaaagttaaattatagatcaataatctatatatcttatctgcag

SEQ ID NO: 6 - protein, 511 aa, Artificial sequence
  Fusion protein consisting of ND4, FLAG tag and Luciferase
MLKIILPSLMLLPLTWLSSPKKTWTNVTSYSFLISLTSLTLLWQTDENYKNFSNIFSSDPLSTPLIILTAWLLPLILIASQNHLKKDNNVLQKLYISILISLQILLIITFSATELIIFYILFEATLIPTLIIITRWGNQTERLNAGIYFLFYTLIGSIPLLIALILIQNHVGTLNLIILSFTTHTLDASWSNNLLWLACIIAFLIKIPLYGVHLWLPKAHVEAPIAGSIILAAILLKLGSYGIIRISIILDPLTKYIAYPFILLSLWGIIITSSICLRQTDLKSLIAYSSVSHIALVIASIIIQTPWSFIGATILIIAHGLTSSLLFCLANSNYERIHSRTIIMARGLQMVFPLIATWWLIASLANLALPPSINLIGELFITISLFSWSNFTIILIGINIIITGIYSIYIIITTQRGKLTNHIINLQPSHTRELTLIALHIIPLILLTTNPKLITGLTIDYKDDDDKMVFTLEDFVGDWRQTAGYNLDQVLEQGGVSSLFQNLGVSVTPIQ

SEQ ID NO: 7 - DNA, 2069 bp, Artificial sequence
  CDS (7)..(1923): Recombinant DNA comprising ND4 coding sequence, FLAG Tag sequence, Luciferase coding sequence and mitochondrial tRNA-Asp sequence
ctgcagatgctaaaaattattcttccctcactaatgctactaccactaacctgactatcaagccctaaaaaaacctgaacaaacgtaacctcatatagttttctaattagtttaaccagcctaacacttctatgacaaaccgacgaaaattataaaaacttttcaaatatattctcctcagaccccctatccacaccattaattattttaacagcctgattactgccactaatattaatagctagccaaaaccacctaaaaaaagataataacgtactacaaaaactctacatctcaatactaatcagcttacaaattctcctaatcataaccttttcagcaactgaactaattatattttatattttatttgaagcaaccttaatcccaacacttattattattacccgatgagggaaccaaactgaacgcctaaacgcagggatttatttcctattttataccctaatcggttctattccactgctaattgccctcatcttaatccaaaaccatgtaggaaccctaaacctcataattttatcattcacaacacacaccttagacgcttcatgatctaacaacttactatggttggcatgcataatagcatttcttattaaaataccattatatggagttcacctatgactaccaaaagcccatgttgaagctccaattgctgggtcaataattctagcagctattcttctaaaattaggtagttacggaataattcgcatctccattattctagacccactaacaaaatatatagcataccccttcatccttctctccctatgaggaataattataactagctcaatctgcttacgccaaacagatttaaaatcactaatcgcctactcctcagttagccacatagcacttgttattgcatcaatcataatccaaactccatgaagcttcataggagcaacaatactaataatcgcacatggcctcacatcatcactcctattctgcctagcaaactccaactacgaacggatccacagccgtactataatcatggcccgaggacttcaaatggtcttcccacttatagccacatgatgactgatagcaagtctagctaatctagctctacccccttcaatcaatctaataggagaattattcattaccatatcattattttcttgatcaaactttaccattattcttataggaattaacattattattacaggtatatactcaatatacataattattaccacccaacgcggcaaactaaccaaccatataattaacctccaaccctcacacacacgagaactaacactaatagcccttcacataattccacttattcttctaactaccaatccaaaactaattacaggcctgacaatagattacaaggatgacgacgataagatggtcttcacactcgaagatttcgttggggactgacgacagacagccggctacaacctggaccaagtccttgaacagggaggtgtgtccagtttgtttcagaatctcggggtgtccgtaactccgatccaacggattgtcctgagcggtgaaaatgggctgaagatcgacatccatgtcatcatcccgtatgaaggtctgagcggcgaccaaatgggccagatcgaaaaaatttttaaggtggtgtaccctgtggatgatcatcactttaaggtgatcctgcactatggcacactggtaatcgacggggttacgccgaacatgatcgactatttcggacggccgtatgaaggcatcgccgtgttcgacggcaaaaagatcactgtaacagggaccctgtggaacggcaacaaaattatcgacgagcgcctgatcaaccccgacggctccctgctgttccgagtaaccatcaacggagtgaccggctggcggctgtgcgaacgcattctggcgtaagaaaggaaggaatcgaaccccctaaaattggtttcaagccaatctcatatcctatatgtctttctcaataagatattagtaaaatcaattacataactttgtcaaagttaaattatagatcaataatctatatatcttatctgcag

SEQ ID NO: 8 - protein, 638 aa, Artificial sequence; identical to SEQ ID NO: 2
  Fusion protein consisting of ND4, FLAG tag and Luciferase

SEQ ID NO: 9 - DNA, 2267 bp, Artificial sequence
  CDS (205)..(2121): Recombinant DNA comprising HSP promoter sequence, ND4 coding sequence, FLAG Tag sequence, Luciferase coding sequence and mitochondrial tRNA-Asp sequence
ctgcagccctcctcttaatgccaaaccccaaaaacactaagaacttgaaagacatataatattaactatcaaaccctatgtcctgatcaattctagtagttcccaaaatatgacttatattttagtacttgtaaaaattttacaaaatcatgttccgtgaaccaaaactctaatcatactctattacgcaataaacattaacaaatgctaaaaattattcttccctcactaatgctactaccactaacctgactatcaagccctaaaaaaacctgaacaaacgtaacctcatatagttttctaattagtttaaccagcctaacacttctatgacaaaccgacgaaaattataaaaacttttcaaatatattctcctcagaccccctatccacaccattaattattttaacagcctgattactgccactaatattaatagctagccaaaaccacctaaaaaaagataataacgtactacaaaaactctacatctcaatactaatcagcttacaaattctcctaatcataaccttttcagcaactgaactaattatattttatattttatttgaagcaaccttaatcccaacacttattattattacccgatgagggaaccaaactgaacgcctaaacgcagggatttatttcctattttataccctaatcggttctattccactgctaattgccctcatcttaatccaaaaccatgtaggaaccctaaacctcataattttatcattcacaacacacaccttagacgcttcatgatctaacaacttactatggttggcatgcataatagcatttcttattaaaataccattatatggagttcacctatgactaccaaaagcccatgttgaagctccaattgctgggtcaataattctagcagctattcttctaaaattaggtagttacggaataattcgcatctccattattctagacccactaacaaaatatatagcataccccttcatccttctctccctatgaggaataattataactagctcaatctgcttacgccaaacagatttaaaatcactaatcgcctactcctcagttagccacatagcacttgttattgcatcaatcataatccaaactccatgaagcttcataggagcaacaatactaataatcgcacatggcctcacatcatcactcctattctgcctagcaaactccaactacgaacggatccacagccgtactataatcatggcccgaggacttcaaatggtcttcccacttatagccacatgatgactgatagcaagtctagctaatctagctctacccccttcaatcaatctaataggagaattattcattaccatatcattattttcttgatcaaactttaccattattcttataggaattaacattattattacaggtatatactcaatatacataattattaccacccaacgcggcaaactaaccaaccatataattaacctccaaccctcacacacacgagaactaacactaatagcccttcacataattccacttattcttctaactaccaatccaaaactaattacaggcctgacaatagattacaaggatgacgacgataagatggtcttcacactcgaagatttcgttggggactgacgacagacagccggctacaacctggaccaagtccttgaacagggaggtgtgtccagtttgtttcagaatctcggggtgtccgtaactccgatccaacggattgtcctgagcggtgaaaatgggctgaagatcgacatccatgtcatcatcccgtatgaaggtctgagcggcgaccaaatgggccagatcgaaaaaatttttaaggtggtgtaccctgtggatgatcatcactttaaggtgatcctgcactatggcacactggtaatcgacggggttacgccgaacatgatcgactatttcggacggccgtatgaaggcatcgccgtgttcgacggcaaaaagatcactgtaacagggaccctgtggaacggcaacaaaattatcgacgagcgcctgatcaaccccgacggctccctgctgttccgagtaaccatcaacggagtgaccggctggcggctgtgcgaacgcattctggcgtaagaaaggaaggaatcgaaccccctaaaattggtttcaagccaatctcatatcctatatgtctttctcaataagatattagtaaaatcaattacataactttgtcaaagttaaattatagatcaataatctatatatcttatctgcag

SEQ ID NO: 10 - protein, 638 aa, Artificial sequence; identical to SEQ ID NO: 2
  Fusion protein consisting of ND4, FLAG tag and Luciferase

SEQ ID NO: 11 - DNA, 2267 bp, Artificial sequence
  CDS (205)..(1740): Recombinant DNA comprising HSP promoter sequence, ND4 coding sequence, FLAG Tag sequence, Luciferase coding sequence and mitochondrial tRNA-Asp sequence
ctgcagccctcctcttaatgccaaaccccaaaaacactaagaacttgaaagacatataatattaactatcaaaccctatgtcctgatcaattctagtagttcccaaaatatgacttatattttagtacttgtaaaaattttacaaaatcatgttccgtgaaccaaaactctaatcatactctattacgcaataaacattaacaaatgctaaaaattattcttccctcactaatgctactaccactaacctgactatcaagccctaaaaaaacctgaacaaacgtaacctcatatagttttctaattagtttaaccagcctaacacttctatgacaaaccgacgaaaattataaaaacttttcaaatatattctcctcagaccccctatccacaccattaattattttaacagcctgattactgccactaatattaatagctagccaaaaccacctaaaaaaagataataacgtactacaaaaactctacatctcaatactaatcagcttacaaattctcctaatcataaccttttcagcaactgaactaattatattttatattttatttgaagcaaccttaatcccaacacttattattattacccgatgagggaaccaaactgaacgcctaaacgcagggatttatttcctattttataccctaatcggttctattccactgctaattgccctcatcttaatccaaaaccatgtaggaaccctaaacctcataattttatcattcacaacacacaccttagacgcttcatgatctaacaacttactatggttggcatgcataatagcatttcttattaaaataccattatatggagttcacctatgactaccaaaagcccatgttgaagctccaattgctgggtcaataattctagcagctattcttctaaaattaggtagttacggaataattcgcatctccattattctagacccactaacaaaatatatagcataccccttcatccttctctccctatgaggaataattataactagctcaatctgcttacgccaaacagatttaaaatcactaatcgcctactcctcagttagccacatagcacttgttattgcatcaatcataatccaaactccatgaagcttcataggagcaacaatactaataatcgcacatggcctcacatcatcactcctattctgcctagcaaactccaactacgaacggatccacagccgtactataatcatggcccgaggacttcaaatggtcttcccacttatagccacatgatgactgatagcaagtctagctaatctagctctacccccttcaatcaatctaataggagaattattcattaccatatcattattttcttgatcaaactttaccattattcttataggaattaacattattattacaggtatatactcaatatacataattattaccacccaacgcggcaaactaaccaaccatataattaacctccaaccctcacacacacgagaactaacactaatagcccttcacataattccacttattcttctaactaccaatccaaaactaattacaggcctgacaatagattacaaggatgacgacgataagatggtcttcacactcgaagatttcgttggggactgacgacagacagccggctacaacctggaccaagtccttgaacagggaggtgtgtccagtttgtttcagaatctcggggtgtccgtaactccgatccaatagattgtcctgagcggtgaaaatgggctgaagatcgacatccatgtcatcatcccgtatgaaggtctgagcggcgaccaaatgggccagatcgaaaaaatttttaaggtggtgtaccctgtggatgatcatcactttaaggtgatcctgcactatggcacactggtaatcgacggggttacgccgaacatgatcgactatttcggacggccgtatgaaggcatcgccgtgttcgacggcaaaaagatcactgtaacagggaccctgtggaacggcaacaaaattatcgacgagcgcctgatcaaccccgacggctccctgctgttccgagtaaccatcaacggagtgaccggctggcggctgtgcgaacgcattctggcgtaagaaaggaaggaatcgaaccccctaaaattggtttcaagccaatctcatatcctatatgtctttctcaataagatattagtaaaatcaattacataactttgtcaaagttaaattatagatcaataatctatatatcttatctgcag

SEQ ID NO: 12 - protein, 511 aa, Artificial sequence; identical to SEQ ID NO: 6
  Fusion protein consisting of ND4, FLAG tag and Luciferase

SEQ ID NO: 13 - protein, 27 aa, Artificial sequence
  KALA peptide
WEAKLAKALAKALAKHLAKALAKALKA